European Patent Application EP 4 140 503 A1, published March 1, 2023. Title: Use of EphB4 as a Target in Screening Drugs or Models for Increasing Insulin Sensitivity. Applicant: INSTITUTE OF MATERIA MEDICA, CHINESE ACADEMY OF MEDICAL SCIENCES. The sequence listing filed with the application follows.

SEQUENCE LISTING (14 sequences)

SEQ ID NO: 1 - DNA, 19 bp, Artificial Sequence
  EphB4 shRNA
gttatgatcctcacggaat

SEQ ID NO: 2 - DNA, 19 bp, Artificial Sequence
  control shRNA
ttctccgaacgtgtcacgt

SEQ ID NO: 3 - DNA, 21 bp, Artificial Sequence
  primer
tatgccacgatacgcttcacc

SEQ ID NO: 4 - DNA, 23 bp, Artificial Sequence
  primer
agcttcgctctcgtaatagaaga

SEQ ID NO: 5 - DNA, 22 bp, Artificial Sequence
  primer
agattcgggatatgctgttggc

SEQ ID NO: 6 - DNA, 21 bp, Artificial Sequence
  primer
tcgggtcctagaccagtgttc

SEQ ID NO: 7 - DNA, 23 bp, Artificial Sequence
  CRISPR-Cas9 targeted sequence 1
gcccgagatctttactccccggg

SEQ ID NO: 8 - DNA, 23 bp, Artificial Sequence
  CRISPR-Cas9 targeted sequence 2
ttctgggctgatcaaagtgtggg

SEQ ID NO: 9 - DNA, 57 bp, Artificial Sequence
  sgRNA sequence 1
ctatttctagctctaaaacggggagtaaagatctcgggcctatagtgagtcgtatta

SEQ ID NO: 10 - DNA, 55 bp, Artificial Sequence
  sgRNA sequence 2
ctatttctagctctaaaacacactttgatcagcccagcctatagtgagtcgtatt

SEQ ID NO: 11 - DNA, 24 bp, Artificial Sequence
  primer
agttcctccaagtcccctaacacc

SEQ ID NO: 12 - DNA, 20 bp, Artificial Sequence
  primer
cgcgcactggtgaaaatccc

SEQ ID NO: 13 - DNA, 22 bp, Artificial Sequence
  primer
ggagaatctggggagtgggaca

SEQ ID NO: 14 - DNA, 25 bp, Artificial Sequence
  primer
actctccttttttgctgggcaaaat